European Patent Application EP 4 400 163 A1, published July 17, 2024. Title: COMPOSITIONS FOR THE TREATMENT OF GLUTEN INTOLERANCE AND USES THEREOF. Applicant: GLUTAGEN PTY LTD. Application EP. The sequence listing filed with the application follows.

SEQUENCE LISTING (12 sequences)

SEQ ID NO: 1 - protein, 348 aa, Carica papaya [sequence omitted]

SEQ ID NO: 2 - protein, 367 aa, Carica papaya
MAMIPSISKLLFVAICLFVHMSVSFGDFSIVGYSQDDLTSTERLIQLFNSWMLNHNKFYENVDEKLYRFEIFKDNLNYIDETNKKNNSYRLGLNEFADLSNDEFNEKYVGSLIDATIEQSYDEEFINEDIVNLPENVDWRKKGAVTPVRHQGSCGSCWAFSAVATVEGINKIRTGKLVELSEQELVDCERRSHGCKGGYPPYALEYVAKNGIHLRSKYPYKAKQGTCRAKQVGGPIVKTSGVGRVQPNNEGNLLNAIAKQPVSVVVESKGRPFQLYKGGIFEGPCGTKVDHAVTAVGYGKSGGKGYILIKNSWGTAWGEKGYIRIKRAPGNSPGVCGLYKSSYYPIKNRDNGRIQIRPSSQHLTSHE

SEQ ID NO: 3 - DNA, 1047 bp, Carica papaya
  source 1..1047: mol_type = genomic DNA
atggctatgataccttcaatttcaaagttgctttttgttgcaatatgtctctttgttcatatgagtgtgtcctttggtgatttttctatcgtggggtattcgcaagatgacttgacatctactgagaggcttattcagctctttaactcgtggatgttgaatcacaataaattttacgagaatgttgatgagaaactttacagatttgaaatttttaaggacaatctaaactacattgacgagacaaacaaaaagaataacagttattggcttggattaaacgagtttgctgatttaagcaatgatgaattcaatgagaagtatgttggttcccttattgatgcaacgattgaacaatcctatgatgaagagtttattaatgaagatactgtaaatttgcccgagaatgtcgattggagaaaaaaaggagctgtcactcccgtaagacatcagggttcatgcggtagttgttgggcattctcggccgttgcaactgtagagggaataaataagattagaactggaaaattagtagaattatcagagcaagaacttgttgactgtgaaagacgtagccatgggtgcaaaggaggttatccgccgtatgcacttgaatatgtggctaagaatggtattcacttgagatcaaagtacccatataaagcaaagcaagggacttgtcgagccaaacaagtgggaggtcccattgtgaaaacttctggggttggacgtgtgcaaccaaataatgaagggaatctcttaaatgcaattgcaaagcaacctgtgagcgttgtggttgaatccaagggaagacctttccaattgtataaagggggaatatttgaggggccatgcggaaccaaagtagatcatgcagtaacagcagttggttatggaaaaagtggaggcaaaggttacatactcatcaagaattcatggggtactgcatggggtgagaaaggatatataagaatcaaaagagcccctggaaactccccaggagtgtgtggactttataaaagctcatactatcctactaaaaattga

SEQ ID NO: 4 - DNA, 1110 bp, Carica papaya
  source 1..1110: mol_type = genomic DNA
atggctatgataccttcaatttcaaagttgctctttgttgcaatatgtctctttgttcatatgagtgtgtcctttggcgatttttctattgtggggtattcgcaagatgacttgacatctaccgagaggcttattcagctctttaactcgtggatgttgaatcacaataaattttacgagaatgttgatgagaaactttacagatttgaaatttttaaggacaatctaaactacattgacgagacaaacaaaaagaataacagttataggcttggattaaacgagtttgctgatttaagcaatgatgaattcaatgagaagtatgttggttcccttattgatgcaacaattgaacaatcctatgatgaagagtttattaatgaagatattgtaaatttgcccgagaatgtcgattggagaaaaaaaggagctgtcactcccgtaagacatcagggttcatgcggtagttgttgggcattctcggccgttgcaactgtagagggaataaataagattagaactggaaaattagtagaattatcagagcaagaacttgttgactgtgaaagacgtagccatgggtgcaaaggaggttatccgccgtatgcacttgaatatgtggctaagaatggtattcacttgagatcaaagtacccatataaagcaaagcaagggacttgtcgagccaaacaagtgggaggtccgattgtgaaaacttctggggttggacgtgtgcaaccaaataatgaagggaatctcttaaatgcaattgcaaagcaacctgtgagcgttgtggttgaatccaagggaagacctttccaattgtataaagggggaatatttgaggggccatgcggaaccaaagtagatcatgcagtaacagcagttggttatggaaaaagtggaggcaaaggttacatactcatcaagaattcatggggtactgcatggggtgagaaaggatatataagaatcaaaagagcccctggaaactccccaggagtgtgtggactttataaaagctcatactatcctattaaaaatagagataatggacggatccagatccgcccatcatctcaacacctcacaagccatgaatgaagctga

SEQ ID NO: 5 - protein, 4 aa, synthetic construct
  REGION 1..4: note = Amino acid motif
PSQQ

SEQ ID NO: 6 - protein, 4 aa, synthetic construct
  REGION 1..4: note = Amino acid motif
QQQP

SEQ ID NO: 7 - protein, 4 aa, synthetic construct
  REGION 1..4: note = Amino acid motif
QQPY

SEQ ID NO: 8 - protein, 9 aa, synthetic construct
  REGION 1..9: note = A-gliadin wheat peptide
QNPSQQQPQ

SEQ ID NO: 9 - protein, 12 aa, synthetic construct
  REGION 1..12: note = A-gliadin wheat peptide
RPQQPYPQPQPQ

SEQ ID NO: 10 - protein, 13 aa, synthetic construct
  REGION 1..13: note = A-gliadin wheat peptide
LGQQQPFPPQQPY

SEQ ID NO: 11 - protein, 12 aa, synthetic construct
  REGION 1..12: note = A-gliadin wheat peptide
PQPQPFPSQQPY

SEQ ID NO: 12 - protein, 12 aa, synthetic construct
  REGION 1..12: note = A-gliadin wheat peptide
LGQGSFRPSQQN